European Patent Specification EP 4 022 071 B1, published October 22, 2025. Title: Method for improving anthocyanin composition in carrots. Applicant: Chr. Hansen A/S. The sequence listing filed with the application follows.

SEQUENCE LISTING (79 sequences)

SEQ ID NO: 1 - DNA, 882 bp, Daucus carota
atgagctattccaagggcatgaagagtgctaacacagcttcaaagctgcgaaagggtgcatgggattttgaggaagacactcttctccgaaaatgcattgacaagtatggagaaggaaagtggcaccttgttccgcagagagctgggttgaatagatgcagaaaaagttgtagactaaggtggcttaactatctgaggcctaccatcaagagaggagaattcagtgctgatgaagtggatcttatgatgcgccttcacaggcttctgggaaaccgatggtcgctgattggaggaagactgccgggaagaacagctaatgatgttaagaactactggaacaccaacattcaaaagaaactcactactcgcagcaacaagaaagacgtggcgataagagaagagcttcttcaaagaaaacaatacagtagtattgctgcaactagtactggtgctactgttataaagcctcttccccggactttatccaaaggcacaagcctatcctgctatgatcttaatcccaagaaacccgttcgtaacttgaatgacacactacacaacaacattaacaacaaggcatcatcaccagcaaaactggcaccgaatgaccaaggcaaggagaccctgccactggatgaagatgtcatagagtggtggaagaatttgtttgaggaaataaacattaatggtcaagagcaagattactcagacggactgttgatggcatcctcgagcggttcagataatgtgcatgctgacagagacttcgtgtggaagacagatgaatcaaccgcagcagcaatggaattgtcagaagatggtttgtgtgacatttggaatcttctagactcatcagaccatgtccgattgagtcggttataa

SEQ ID NO: 2 - DNA, 1785 bp, Daucus carota
atggcagagatcctgagaaagcagctggctcttgctgttaagaagattcagtggagctatgcaattttctgggccatttcatcatcacagaatggggtattggagtgggatgatgggtactacaatggagatataaagacgcgaaaaacagttcaagcagaacagttaaatgttgatcagcttggattacaaaggactgagcaattgagagaactttatgagtccctcctggatgccgaaaacaacagacactctgcaaggccttctgctgcattatctcctgaagatcttactgataccgagtggtatttcttgatatgcatgtcgtttgtgttcaatagtggccaagggttgcctgggagatcattagcaaaaaatcaaaccacttggttgtgcaatgcaaattatgcagatagcaaagtgtttaatcgtgttctgcttgcaaagagtgcattgattcagacagttgtatgctttccatattcagatggcgtaattgaaattggtacaactgacctggtttcagaggatcctagtatagtccagtacataaaatctttcttggggactccaggggcaatttttgagagtgttgctgatgccgatctgaacccagatactgaatgggaaaaaggcaacatgtgctcctcaaatggtagtttagaagaagttgagccaaattatcaggcaaaggaatcactagtggctgaacgccttgatgatggcacctctcagcaaaaaagctggcaattaatggatggtgaaatcagtaacactttcctcgactctggagattccagtgactgtatatccgaaacctttatagcccctgaaaagactgtccctcaacaagataaatataacaaggttgatgaaaaccgtctacttgagcttcaaggttccaaggatatggaactgacttcagttgagattctggaagatgatttcaactaccaaggtattgtgtccacccttctgaagacttcccaccaattgattatgggaccatgtttcaaaagcagtataaaagattcatgctttgttagatggaaaaaaggcagatccccgtgtaaatacaagtcaggtggaacttctcaaagattgctgaaaaaggtactgtacgaagttcctgtaaagcataacgatggtaaaataaggaaaccagagagttttgaatctgatacaaaccatgcaccagaagagagaaggcaaagagaaaagatgcaggaaaagtttatgattcttagatcgatagtaccttcaactggcaaggttgacaatgtgtcattgcttgatgagactatagaataccttagaaatcttgagaaaagggttgagggattagaatctcagaaagagcttgtagacgtagaagcaagaaggggaaagagaatttttaatgtcatagagagtacttctgataactatggcgacatgagagtaagttacagcaagaagcaggtgctgaataagaggaagggttctggtaccaacactatgaatgctataaaccaattgcatcaggaagacaataagactgacgacgtgaaagtttctaaaacagggaagggcattgtcatagagattgaatgtccttggcgagaggagttgtttgtagatatcatgggcgcaataaacaaccttcatttggattctcactcggttcaatcttccaagattgatggaaacctttctttgacgattaactctaaggtgaaaggatcaactatgccatctgtaaatataataagacaagcacttcaacgagttaccagaaagtcctaa

SEQ ID NO: 3 - DNA, 436 bp, Cauliflower mosaic virus
ctcgagatccgtcaacatggtggagcacgacactctcgtctactccaagaatatcaaagatacagtctcagaagaccaaagggctattgagacttttcaacaaagggtaatatcgggaaacctcctcggattccattgcccagctatctgtcacttcatcaaaaggacagtagaaaaggaaggtggcacctacaaatgccatcattgcgataaaggaaaggctatcgttcaagatgcctctgccgacagtggtcccaaagatggacccccacccacgaggagcatcgtggaaaaagaagacgttccaaccacgtcttcaaagcaagtggattgatgtgatatctccactgacgtaagggatgacgcacaatcccactatccttcgcaagacccttcctctatataaggaagttcatttcatttggagaggacgacc

SEQ ID NO: 4 - DNA, 1422 bp, Daucus carota
atgagccctgtatatcaagactccaaaaaggatcttgttcatatcttacttgtgtctttcataggacaaggccatgtcaaccctttactcagactaggaaacctccttgcttcatcaggtttccttgtcaccttctcttcctgttcggaagtcggaaattccatgcgcaaggctaacaacaacatcgatgaactcgttccagttggcgatgggatgatcaggtttgagttttttgatgatggattacccgagagtgatccacgacgccatgatctcgacttctacatgcctcaccttgagttgcatggtaaagaggcagtcactggcattgtcaagaaacacgaaaaagaagggcgtccggtgtcatgcatcatcaacaatcctttcattccatgggtttctgacatcgcggaggccttaagcattcgtaatgcagtgctttgggtacagtcctgtgcttgtttttcagcttattaccattaccacaataagttgtcacagtttccctccgaatctgaacccgaaatcgatgtccaactgccatctatgcctctgttaaaacatgatgaaatcccaagtttcttacacccttcaactccttatccagccttaagaagaacaattctagcccaattcaagaacttgtcaaaaccattctgtgtactagtagaaacatttcaagaactcgaaagtgaagtcattgattacatgtccaaactctgccccatcaaggccatcggccctctattcaagaacccgaaatctcaactttctaacatccaaggcgattgcttgaagcccgtcgatgactgcatcgatttcctgaactccaaaagcccctcatccgttgtctacatctctttcggcagtgttatctcaatgaaccaaaaacaaacaaatgaacttgctcaaggtcttttaaactccggagtttcttttctctgggtttttaggccaccccttccaggtttcgacgtagctgtactacccgaaaaattcctggaagcagctggtgacaagggaaaagtagtgcagtggtgttcacagaaacaagtcctggcaagtcctgcagtggcttgttttctgacacattgcggatggaattcgacgttagaggccttaacaactggtgtccctgtgataacctaccctgcatggggtgatcaagtcactaatgctaagtttttagttgatgtgttaaaagtgggagtcaggttaagtagagggaaccaatctaaaaaaaatgtcatttccagggacgatatcgaaaaatctttaagagaagctaccattggggaaaatgcagcagagattaaaaggaatgcattgaagtggaaggaggcggcagaggacgcggtggcagagggcggttcttctgatcggaacttgaaagagtttgtggataagctgatgatgaactga

SEQ ID NO: 5 - protein, 293 aa, Daucus carota
MSYSKGMKSANTASKLRKGAWDFEEDTLLRKCIDKYGEGKWHLVPQRAGLNRCRKSCRLRWLNYLRPTIKRGEFSADEVDLMMRLHRLLGNRWSLIGGRLPGRTANDVKNYWNTNIQKKLTTRSNKKDVAIREELLQRKQYSSIAATSTGATVIKPLPRTLSKGTSLSCYDLNPKKPVRNLNDTLHNNINNKASSPAKLAPNDQGKETLPLDEDVIEWWKNLFEEININGQEQDYSDGLLMASSSGSDNVHADRDFVWKTDESTAAAMELSEDGLCDIWNLLDSSDHVRLSRL

SEQ ID NO: 6 - protein, 594 aa, Daucus carota
MAEILRKQLALAVKKIQWSYAIFWAISSSQNGVLEWDDGYYNGDIKTRKTVQAEQLNVDQLGLQRTEQLRELYESLLDAENNRHSARPSAALSPEDLTDTEWYFLICMSFVFNSGQGLPGRSLAKNQTTWLCNANYADSKVFNRVLLAKSALIQTVVCFPYSDGVIEIGTTDLVSEDPSIVQYIKSFLGTPGAIFESVADADLNPDTEWEKGNMCSSNGSLEEVEPNYQAKESLVAERLDDGTSQQKSWQLMDGEISNTFLDSGDSSDCISETFIAPEKTVPQQDKYNKVDENRLLELQGSKDMELTSVEILEDDFNYQGIVSTLLKTSHQLIMGPCFKSSIKDSCFVRWKKGRSPCKYKSGGTSQRLLKKVLYEVPVKHNDGKIRKPESFESDTNHAPEERRQREKMQEKFMILRSIVPSTGKVDNVSLLDETIEYLRNLEKRVEGLESQKELVDVEARRGKRIFNVIESTSDNYGDMRVSYSKKQVLNKRKGSGTNTMNAINQLHQEDNKTDDVKVSKTGKGIVIEIECPWREELFVDIMGAINNLHLDSHSVQSSKIDGNLSLTINSKVKGSTMPSVNIIRQALQRVTRKS

SEQ ID NO: 7 - protein, 473 aa, Daucus carota
MSPVYQDSKKDLVHILLVSFIGQGHVNPLLRLGNLLASSGFLVTFSSCSEVGNSMRKANNNIDELVPVGDGMIRFEFFDDGLPESDPRRHDLDFYMPHLELHGKEAVTGIVKKHEKEGRPVSCIINNPFIPWVSDIAEALSIRNAVLWVQSCACFSAYYHYHNKLSQFPSESEPEIDVQLPSMPLLKHDEIPSFLHPSTPYPALRRTILAQFKNLSKPFCVLVETFQELESEVIDYMSKLCPIKAIGPLFKNPKSQLSNIQGDCLKPVDDCIDFLNSKSPSSVVYISFGSVISMNQKQTNELAQGLLNSGVSFLWVFRPPLPGFDVAVLPEKFLEAAGDKGKVVQWCSQKQVLASPAVACFLTHCGWNSTLEALTTGVPVITYPAWGDQVTNAKFLVDVLKVGVRLSRGNQSKKNVISRDDIEKSLREATIGENAAEIKRNALKWKEAAEDAVAEGGSSDRNLKEFVDKLMMN

SEQ ID NO: 8 - DNA, 23 bp, Artificial Sequence
  PCR primer
atgagctattccaagggcatgaa

SEQ ID NO: 9 - DNA, 22 bp, Artificial Sequence
  PCR primer
atggcagagatcctgagaaagc

SEQ ID NO: 10 - DNA, 26 bp, Artificial Sequence
  PCR primer
atgcattcaaagggtatgaagattac

SEQ ID NO: 11 - DNA, 27 bp, Artificial Sequence
  PCR primer
tcaactatagtcctggttcagaagatc

SEQ ID NO: 12 - DNA, 27 bp, Artificial Sequence
  PCR primer
atgaagaattgtaatcctttgaaggtg

SEQ ID NO: 13 - DNA, 32 bp, Artificial Sequence
  PCR primer
ttaaatgtaatctaagttgagaagattccaaa

SEQ ID NO: 14 - DNA, 24 bp, Artificial Sequence
  PCR primer
ttataaccgactcaatcggacatg

SEQ ID NO: 15 - DNA, 25 bp, Artificial Sequence
  PCR primer
ttaggactttctggtaactcgttga

SEQ ID NO: 16 - DNA, 20 bp, Artificial Sequence
  PCR primer
atggcttcaccaccacctta

SEQ ID NO: 17 - DNA, 27 bp, Artificial Sequence
  PCR primer
ctccatctgaattaacctagtaactca

SEQ ID NO: 18 - DNA, 50 bp, Artificial Sequence
  PCR primer
gaattctgatctgagacccggacgtgggcaggtggtgttgacaattaatc

SEQ ID NO: 19 - DNA, 37 bp, Artificial Sequence
  PCR primer
attttgccgtcaaggcgatatcgacaaaggaaaaggg

SEQ ID NO: 20 - DNA, 34 bp, Artificial Sequence
  PCR primer
cttttcctttgtcgatatcaaatcccttaacgtg

SEQ ID NO: 21 - DNA, 48 bp, Artificial Sequence
  PCR primer
gatctcgaggatcatgagcaggtgcgcaggaaagaacatgtgagcaaa

SEQ ID NO: 22 - DNA, 33 bp, Artificial Sequence
  PCR primer
cacctgctcatgatcctcgagatccgtcaacat

SEQ ID NO: 23 - DNA, 34 bp, Artificial Sequence
  PCR primer
ggtgcctgagaccggtcgtcctctccaaatgaaa

SEQ ID NO: 24 - DNA, 40 bp, Artificial Sequence
  PCR primer
gaccggtctcaggcaccatgagctattccaagggcatgaa

SEQ ID NO: 25 - DNA, 39 bp, Artificial Sequence
  PCR primer
gcttggtctcagtcgttataaccgactcaatcggacatg

SEQ ID NO: 26 - DNA, 33 bp, Artificial Sequence
  PCR primer
acgatcggggaaattcaagcttggtctcagtcg

SEQ ID NO: 27 - DNA, 39 bp, Artificial Sequence
  PCR primer
cacctgcccacgtccggaattcgtcaccgggcgatctag

SEQ ID NO: 28 - DNA, 38 bp, Artificial Sequence
  PCR primer
gaattccccggtgacgcaggtggtgttgacaattaatc

SEQ ID NO: 29 - DNA, 46 bp, Artificial Sequence
  PCR primer
ctcgagggtcccctggcaggtgcgcaggaaagaacatgtgagcaaa

SEQ ID NO: 30 - DNA, 34 bp, Artificial Sequence
  PCR primer
cacctgccaggggaccctcgagatccgtcaacat

SEQ ID NO: 31 - DNA, 41 bp, Artificial Sequence
  PCR primer
ggtccaatgagacctctagaggtcgtcctctccaaatgaaa

SEQ ID NO: 32 - DNA, 45 bp, Artificial Sequence
  PCR primer
acctctagaggtctcattggaccatggcagagatcctgagaaagc

SEQ ID NO: 33 - DNA, 47 bp, Artificial Sequence
  PCR primer
attcggtctcaccatagtcgacttaggactttctggtaactcgttga

SEQ ID NO: 34 - DNA, 34 bp, Artificial Sequence
  PCR primer
gtcgactatggtgagaccgaatttccccgatcgt

SEQ ID NO: 35 - DNA, 41 bp, Artificial Sequence
  PCR primer
cacctgcgtcaccggggaattccgatctagtaacatagatg

SEQ ID NO: 36 - DNA, 70 bp, Artificial Sequence
  PCR primer
taatacgactcactatatccggatcaaaagcaggtgatgttctttcctgcgttatcccctgattctgtgg

SEQ ID NO: 37 - DNA, 49 bp, Artificial Sequence
  PCR primer
ctcctcgcccttgctcaccatggtataagctgtttcctgtgtgaaattg

SEQ ID NO: 38 - DNA, 37 bp, Artificial Sequence
  PCR primer
ggaaacagcttataccatggtgagcaagggcgaggag

SEQ ID NO: 39 - DNA, 56 bp, Artificial Sequence
  PCR primer
ggaacaaaagctggagctccggtgacgcaggtgttacttgtacagctcgtccatgc

SEQ ID NO: 40 - DNA, 21 bp, Artificial Sequence
  PCR primer
cacacggtgccaatttatgaa

SEQ ID NO: 41 - DNA, 18 bp, Artificial Sequence
  PCR primer
gatcacggccagcaaggt

SEQ ID NO: 42 - DNA, 20 bp, Artificial Sequence
  PCR primer
aaggcacaagcctatcctgc

SEQ ID NO: 43 - DNA, 20 bp, Artificial Sequence
  PCR primer
tggtcattcggtgccagttt

SEQ ID NO: 44 - DNA, 24 bp, Artificial Sequence
  PCR primer
tggagatataaagacgcgaaaaac

SEQ ID NO: 45 - DNA, 19 bp, Artificial Sequence
  PCR primer
ggcatccaggagggactca

SEQ ID NO: 46 - DNA, 22 bp, Artificial Sequence
  PCR primer
ctggcatggcctctatggtact

SEQ ID NO: 47 - DNA, 22 bp, Artificial Sequence
  PCR primer
tgtcctggatggtgcttcaact

SEQ ID NO: 48 - DNA, 19 bp, Artificial Sequence
  PCR primer
gtggaggccaacggaaatg

SEQ ID NO: 49 - DNA, 21 bp, Artificial Sequence
  PCR primer
cgtccgattgtgataccgaga

SEQ ID NO: 50 - DNA, 21 bp, Artificial Sequence
  PCR primer
aaacacctgccgttacactcg

SEQ ID NO: 51 - DNA, 23 bp, Artificial Sequence
  PCR primer
cggaagcaagatcatcatcgtat

SEQ ID NO: 52 - DNA, 23 bp, Artificial Sequence
  PCR primer
ttccaccttctcaaagatgttcc

SEQ ID NO: 53 - DNA, 24 bp, Artificial Sequence
  PCR primer
gctcaactctgtttcaacttggtc

SEQ ID NO: 54 - DNA, 19 bp, Artificial Sequence
  PCR primer
tcctgccacggtcaaacct

SEQ ID NO: 55 - DNA, 19 bp, Artificial Sequence
  PCR primer
aagagcgagcgacggaatc

SEQ ID NO: 56 - DNA, 25 bp, Artificial Sequence
  PCR primer
gagtacagtgagaagctgatgggtc

SEQ ID NO: 57 - DNA, 21 bp, Artificial Sequence
  PCR primer
ggttgagggcacttgggatag

SEQ ID NO: 58 - DNA, 21 bp, Artificial Sequence
  PCR primer
ttgaggatggtgaaggtggga

SEQ ID NO: 59 - DNA, 19 bp, Artificial Sequence
  PCR primer
cttttgggcgacgcagaac

SEQ ID NO: 60 - DNA, 23 bp, Artificial Sequence
  PCR primer
gttatcaagcctaccgtacaggg

SEQ ID NO: 61 - DNA, 24 bp, Artificial Sequence
  PCR primer
agttccagcagacgaagtgtaaat

SEQ ID NO: 62 - DNA, 22 bp, Artificial Sequence
  PCR primer
aggtgcccacagtcgacatagc

SEQ ID NO: 63 - DNA, 20 bp, Artificial Sequence
  PCR primer
cgcctgtccagccactctaa

SEQ ID NO: 64 - DNA, 23 bp, Artificial Sequence
  PCR primer
attcgaggaactagaccctgacc

SEQ ID NO: 65 - DNA, 24 bp, Artificial Sequence
  PCR primer
gccacagacttaggattacgcttg

SEQ ID NO: 66 - DNA, 28 bp, Artificial Sequence
  PCR primer
ttgatccccctcgagatccgtcaacatg

SEQ ID NO: 67 - DNA, 32 bp, Artificial Sequence
  PCR primer
caattcttttccatggtcgtcctctccaaatg

SEQ ID NO: 68 - DNA, 34 bp, Artificial Sequence
  PCR primer
gaggacgaccatggaaaagaattgtcgtggagtg

SEQ ID NO: 69 - DNA, 38 bp, Artificial Sequence
  PCR primer
gggaaattcaagcttttaatttccaatttgttgggcct

SEQ ID NO: 70 - DNA, 34 bp, Artificial Sequence
  PCR primer
tggaaattaaaagcttgaatttccccgatcgttc

SEQ ID NO: 71 - DNA, 33 bp, Artificial Sequence
  PCR primer
ggctgcaggaattccgatctagtaacatagatg

SEQ ID NO: 72 - DNA, 32 bp, Artificial Sequence
  PCR primer
aagcttgatatcgaattcgatccgtcaacatg

SEQ ID NO: 73 - DNA, 37 bp, Artificial Sequence
  PCR primer
ttggagaggacgaccatggctactggtatccaaaacc

SEQ ID NO: 74 - DNA, 37 bp, Artificial Sequence; identical to SEQ ID NO: 73
  PCR primer

SEQ ID NO: 75 - DNA, 45 bp, Artificial Sequence
  PCR primer
gggaaattctctagatcaagacttcataataactttctgaagagc

SEQ ID NO: 76 - DNA, 42 bp, Artificial Sequence
  PCR primer
gttattatgaagtcttgatctagagaatttccccgatcgttc

SEQ ID NO: 77 - DNA, 38 bp, Artificial Sequence
  PCR primer
gaacaaaagctggagctcccgatctagtaacatagatg

SEQ ID NO: 78 - DNA, 33 bp, Artificial Sequence
  PCR primer
ctagatcggaattcctgcaggatccgtcaacat

SEQ ID NO: 79 - DNA, 32 bp, Artificial Sequence
  PCR primer
gatcccccgggctgcaggaattccgatctagt